European Patent Application EP 4 389 883 A1, published June 26, 2024. Title: POLYMER SUBSTRATE-ENZYME COMPLEX. Applicant: Helmut Schwab. The sequence listing filed with the application follows.

SEQUENCE LISTING (7 sequences)

SEQ ID NO: 1 - protein, 494 aa, Acidovorax sp.
MAFNFIRAAAAGAAMALCGAGGVHAAVNLPALKIDKTQTTVSGLSSGGFMAVQLHVAYSATFAKGAGVVAGGPFYCAEGSIVNATGRCMASPAGIPTSTLVSTTNTWASQGVIDPVANLQTSKVYLFSGTLDSVVKTGVMDALRTYYNSFVPAANVVYKKDIAAEHAMVTDDYGNACSTKGAPYISDCNFDLAGAMLQHLYGTLNARNNATLPTGNYIEFNQSEFITNHGMATTGWAYVPQACQAGGTATCKLHVVLHGCKQNISDVQQQYVRNTGYNRWADTNNIVMLYPQTSTAATNSCWDWWGYDSANYSKKSGPQMAAIKAMVDRVSSGTGGTTPPDPVALPAPTGVSTSGATASSMAIGWAAVTGAASYNVYRNANKVNALPVTATSYTDTGLAASTTYSWTVRAADANGAEGATSAAASGTTLAASGGGTATCTTASNYAHTLAGRAYAAGGYTYALGSNQNMGLWNVFVTNTLKQTSTNYYVIGTCP

SEQ ID NO: 2 - protein, 469 aa, Acidovorax sp.
AVNLPALKIDKTQTTVSGLSSGGFMAVQLHVAYSATFAKGAGVVAGGPFYCAEGSIVNATGRCMASPAGIPTSTLVSTTNTWASQGVIDPVANLQTSKVYLFSGTLDSVVKTGVMDALRTYYNSFVPAANVVYKKDIAAEHAMVTDDYGNACSTKGAPYISDCNFDLAGAMLQHLYGTLNARNNATLPTGNYIEFNQSEFITNHGMATTGWAYVPQACQAGGTATCKLHVVLHGCKQNISDVQQQYVRNTGYNRWADTNNIVMLYPQTSTAATNSCWDWWGYDSANYSKKSGPQMAAIKAMVDRVSSGTGGTTPPDPVALPAPTGVSTSGATASSMAIGWAAVTGAASYNVYRNANKVNALPVTATSYTDTGLAASTTYSWTVRAADANGAEGATSAAASGTTLAASGGGTATCTTASNYAHTLAGRAYAAGGYTYALGSNQNMGLWNVFVTNTLKQTSTNYYVIGTCP

SEQ ID NO: 3 - protein, 507 aa, synthetic construct
  source 1..507: note = as SEQ ID No. 1 plus C-terminal His-tag
MAFNFIRAAAAGAAMALCGAGGVHAAVNLPALKIDKTQTTVSGLSSGGFMAVQLHVAYSATFAKGAGVVAGGPFYCAEGSIVNATGRCMASPAGIPTSTLVSTTNTWASQGVIDPVANLQTSKVYLFSGTLDSVVKTGVMDALRTYYNSFVPAANVVYKKDIAAEHAMVTDDYGNACSTKGAPYISDCNFDLAGAMLQHLYGTLNARNNATLPTGNYIEFNQSEFITNHGMATTGWAYVPQACQAGGTATCKLHVVLHGCKQNISDVQQQYVRNTGYNRWADTNNIVMLYPQTSTAATNSCWDWWGYDSANYSKKSGPQMAAIKAMVDRVSSGTGGTTPPDPVALPAPTGVSTSGATASSMAIGWAAVTGAASYNVYRNANKVNALPVTATSYTDTGLAASTTYSWTVRAADANGAEGATSAAASGTTLAASGGGTATCTTASNYAHTLAGRAYAAGGYTYALGSNQNMGLWNVFVTNTLKQTSTNYYVIGTCPKLAAALEHHHHHH

SEQ ID NO: 4 - protein, 10 aa, synthetic construct
  source 1..10: note = enzyme motif
  VARIANT 5: note = X is threonine, serine, glycine, glutamic acid, glutamine or aspartic acid
ANLQXSKVYL

SEQ ID NO: 5 - protein, 10 aa, synthetic construct
  source 1..10: note = enzyme motif
ANLQNSKVYL

SEQ ID NO: 6 - protein, 10 aa, synthetic construct
  source 1..10: note = enzyme motif
GATANSMAIG

SEQ ID NO: 7 - protein, 12 aa, synthetic construct
  source 1..12: note = enzyme motif
SGATANSMAIGW